European Patent Application EP 4 512 422 A2, published February 26, 2025. Title: HOMOGENEOUS ANTIBODY POPULATIONS. Applicant: AMGEN INC. Application EP, filed September 11, 2008. The sequence listing filed with the application follows.

SEQUENCE LISTING (86 sequences)

SEQ ID NO: 1 - protein, 15 aa, Homo sapiens
EPKSCDKTHTCPPCP

SEQ ID NO: 2 - protein, 12 aa, Homo sapiens
ERKCCVECPPCP

SEQ ID NO: 3 - protein, 61 aa, Homo sapiens
ELKTPLDTTHTCPRCPEPKSCDTPPPCPRCPEPKSCDTPPPCPRCPEPKSCDTPPPCPRCP

SEQ ID NO: 4 - protein, 12 aa, Homo sapiens
ESKYGPPCPSCP

SEQ ID NO: 5 - protein, 17 aa, Homo sapiens
KCCVECPPCPAPPVAGP

SEQ ID NO: 6 - protein, 21 aa, Homo sapiens
KSCDKTHTCPPCPAPELLGGP

SEQ ID NO: 7 - protein, 10 aa, Homo sapiens
KCCVECPPCP

SEQ ID NO: 8 - protein, 10 aa, Homo sapiens
KSCVECPPCP

SEQ ID NO: 9 - protein, 10 aa, Homo sapiens
KCSVECPPCP

SEQ ID NO: 10 - protein, 10 aa, Homo sapiens
KSSVECPPCP

SEQ ID NO: 11 - protein, 26 aa, Homo sapiens
CCVECPPCPAPPVAGPSVFLFPPKPK

SEQ ID NO: 12 - protein, 12 aa, Homo sapiens
GPSVFPLAPCSR

SEQ ID NO: 13 - protein, 10 aa, Homo sapiens
RKCCVECPPC

SEQ ID NO: 14 - protein, 11 aa, Homo sapiens
  VARIANT 4: note = Xaa = Any Amino Acid
  VARIANT 4: note = Xaa = Any Amino Acid
RKCXCVECPPC

SEQ ID NO: 15 - protein, 12 aa, Homo sapiens
  VARIANT 4..5: note = Xaa = Any Amino Acid
RKCXXCVECPPC

SEQ ID NO: 16 - protein, 13 aa, Homo sapiens
  VARIANT 4..6: note = Xaa = Any Amino Acid
RKCXXXCVECPPC

SEQ ID NO: 17 - protein, 12 aa, Homo sapiens
  VARIANT 3: note = Xaa = Any Amino Acid
  VARIANT 5: note = Xaa is any amino acid
RKXCXCVECPPC

SEQ ID NO: 18 - protein, 13 aa, Homo sapiens
  VARIANT 3: note = Xaa = Any Amino Acid
  VARIANT 5..6: note = Xaa = Any Amino Acid
RKXCXXCVECPPC

SEQ ID NO: 19 - protein, 13 aa, Homo sapiens
  VARIANT 3..4: note = Xaa = Any Amino Acid
  VARIANT 6: note = Xaa = Any Amino Acid
RKXXCXCVECPPC

SEQ ID NO: 20 - protein, 14 aa, Homo sapiens
  VARIANT 3..4: note = Xaa = Any Amino Acid
  VARIANT 6..7: note = Xaa = Any Amino Acid
RKXXCXXCVECPPC

SEQ ID NO: 21 - protein, 11 aa, Homo sapiens
  VARIANT 3: note = Xaa = Any Amino Acid
  VARIANT 3: note = Xaa = Any Amino Acid
RKXCCVECPPC

SEQ ID NO: 22 - protein, 12 aa, Homo sapiens
  VARIANT 3..4: note = Xaa = Any Amino Acid
RKXXCCVECPPC

SEQ ID NO: 23-25 - skipped (3 entries)

SEQ ID NO: 26 - protein, 5 aa, Homo sapiens
  VARIANT 4: note = Xaa = Any Amino Acid
  VARIANT 4: note = Xaa = Any Amino Acid
GECXS

SEQ ID NO: 27 - protein, 6 aa, Homo sapiens
  VARIANT 4..5: note = Xaa = Any Amino Acid
GECXXS

SEQ ID NO: 28 - protein, 7 aa, Homo sapiens
  VARIANT 4..6: note = Xaa = Any Amino Acid
GECXXXS

SEQ ID NO: 29 - protein, 5 aa, Homo sapiens
  VARIANT 5: note = Xaa = Any Amino Acid
  VARIANT 5: note = Xaa = Any Amino Acid
GECSX

SEQ ID NO: 30 - protein, 6 aa, Homo sapiens
  VARIANT 5..6: note = Xaa = Any Amino Acid
GECSXX

SEQ ID NO: 31 - protein, 7 aa, Homo sapiens
  VARIANT 5..7: note = Xaa = Any Amino Acid
GECSXXX

SEQ ID NO: 32 - protein, 9 aa, Homo sapiens
CACVECPPC

SEQ ID NO: 33 - protein, 10 aa, Homo sapiens
CPPCVECPPC

SEQ ID NO: 34 - protein, 98 aa, Homo sapiens
VSGGSINSGDYYWSWIRQHPGKGLDCIGYIYYSGSTYYNPSLKSRVTISVDTSKNQFFLKLTSVTAADTAVYYCARSTVVNPGWFDPWGQGTLVTVSS

SEQ ID NO: 35 - protein, 105 aa, Homo sapiens
TITCQASQDINNYLNWFQQKPGKAPKVLIHDASNLETGGPSRFSGSGSGTDFTFTISGLQPEDIATYYCQQYESLPLTFGGGTKVEIKRTVAAPSVFIFPPSDEQ

SEQ ID NO: 36 - protein, 97 aa, Homo sapiens
VSGGSINSGDYYWSWIRQHPGKGLEWIGSIYYSGNTFYNPSLKSRVTISLDTSKNQFSLKLSSVTAADTAVCYCARNIVTTGAFDIWGQGTMVTVSS

SEQ ID NO: 37 - protein, 105 aa, Homo sapiens
TITCQASQDITIYLNWYQQKPGKAPKLLINDASSLETGVPLRFSGSGSGTDFTFTISSLQPEDIATYYCQQYDHLPLTFGGGTKVAIKRTVAAPSVFIFPPSDEQ

SEQ ID NO: 38 - protein, 96 aa, Homo sapiens
VSGGSISSGDYYWTWIRQHPGKGLEWIGYIYYSGNTYYNPSLKSRVSMSIDTSENQFSLKLSSVTAADTAVYYCARKPVTGGEDYWGQGTLVTVSS

SEQ ID NO: 39 - protein, 105 aa, Homo sapiens
TITCQASQDISNYLNWYQQKPGKAPKLLIYDASNLETGVPSRFSGSGSGTDFTFTISSLQPEDIVGYYVQQYESLPCGFGQGTKLEIKRTVAAPSVFIFPPSDEQ

SEQ ID NO: 40 - protein, 97 aa, Homo sapiens
VSGGSINSGDFYWSWIRQHPGKGLEWIGYIYYSGSTYYNPSLKSRVTMSIDPSKNQFSLKLISVTAADTAVYYCATSLYYGGGMDVWGQGTTVTVSS

SEQ ID NO: 41 - protein, 105 aa, Homo sapiens
  VARIANT 87: note = Xaa = Any Amino Acid
TITCQASQDISNNLNWYQQKRGNAPKLLIYDASNLETGVPSRFSGSGSGTDFTFTISNLQPEDIATYYCQHYDHLPWTFGQGTKVEXKRTVAAPSVFIFPPSDEQ

SEQ ID NO: 42 - protein, 97 aa, Homo sapiens
VSGGSINNGDYYWSWIRQHPGKGLEWIGHIYYSGSTYYIPSLKSRTTISVDTSKNQFSLKLNSVTAADTAVYYCARGTVTTYYFDYWGQGTTVTVSS

SEQ ID NO: 43 - protein, 107 aa, Homo sapiens
TITCRASQSISSYLNWYQQKPGKAPKLLIYAASSLQSGVPSRFSGSGSGTDFTLTISSLQPEDFATYYCQQGYRTPPECSFGQGTKLEIKRTVAAPSVFIFPPSDEQ

SEQ ID NO: 44 - protein, 97 aa, Homo sapiens
VSGGSVSSGDYYWSWIRQPPGKGLEWIGHLYYSGNTNYNPSLKSRVTISLDTSKNQFSLKLSSVTAADTAVYYCARDFLTGSFFDYWGQGTLVTVSS

SEQ ID NO: 45 - protein, 105 aa, Homo sapiens
TITCQASQDISNYLNWYQQKPGKAPKLLINDASDLETGVPSRISGSGSGTDFTFTISNLQPEDIATYYCQQYDSLPLTFGGGTKVEIRRTVAAPSVFIFPPSDEQ

SEQ ID NO: 46 - protein, 96 aa, Homo sapiens
VSGGSVYSGDYYWSWIRQPPGKGLEWIGYIYYSGSTNYNPSLKSRVTISVDTSKNQFSLKLSSVTAADTAVYYCARDSILGATNYWGQGTLVTVSS

SEQ ID NO: 47 - protein, 105 aa, Homo sapiens
  VARIANT 9: note = Xaa = Any Amino Acid
  VARIANT 15: note = Xaa = Any Amino Acid
  VARIANT 27: note = Xaa = Any Amino Acid
  VARIANT 51..52: note = Xaa = Any Amino Acid
  VARIANT 70: note = Xaa = Any Amino Acid
  VARIANT 73: note = Xaa = Any Amino Acid
TITCQASQXISNYLXWYQQKPGKAPKXLISDASNLETGVPSRFSGSGSGTXXTFTISSLQPEDIATYHCXQYXSLPLTFGGGTKVEIKRTVAAPSVFIFPPSDEQ

SEQ ID NO: 48 - protein, 95 aa, Homo sapiens
VSGGSVSSGDYYWTWIRQSPGKGLEWIGHIYYSGNTNYNPSLKSRLTISIDTSKTQFSLKLSSVTAADTAIYYCVRDRVTGAFDIWGQGTMVTSS

SEQ ID NO: 49 - protein, 105 aa, Homo sapiens
TITCQASQDISNYLNWYQQKPGKAPKLLIYDASNLETGVPSRFSGSGSGTDFTFTISSLQPEDIATYFCQHFDHLPLAFGGGTKVEIKRTVAAPSVFIFPPSDEQ

SEQ ID NO: 50 - protein, 119 aa, Homo sapiens
VSGGSINSGDYYWSWIRQHPGKGLDCIGYIYYSGSTYYNPSLKSRVTISVDTSKNQFFLKLTSVTAADTAVYYCARSTVVNPGWFDPWGQGTLVTVSSASTKGPSVFPPLAPCSRSTST

SEQ ID NO: 51 - protein, 118 aa, Homo sapiens
VSGGSINSGDYYWSWIRQHPGKGLEWIGSIYYSGNTFYNPSLKSRVTISLDTSKNQFSLKLSSVTAADTAVCYCARNIVTTGAFDIWGQGTMVTVSSASTKGPSVFPPLAPCSRSTST

SEQ ID NO: 52 - protein, 117 aa, Homo sapiens
VSGGSISSGDYYWTWIRQHPGKGLEWIGYIYYSGNTYYNPSLKSRVSMSIDTSENQFSLKLSSVTAADTAVYYCARKPVTGGEDYWGQGTLVTVSSASTKGPSVFPPLAPCSRSTST

SEQ ID NO: 53 - protein, 118 aa, Homo sapiens
VSGGSINSGDFYWSWIRQHPGKGLEWIGYIYYSGSTYYNPSLKSRVTMSIDPSKNQFSLKLISVTAADTAVYYCATSLYYGGGMDVWGQGTTVTVSSASTKGPSVFPPLAPCSRSTST

SEQ ID NO: 54 - protein, 118 aa, Homo sapiens
VSGGSINNGDYYWSWIRQHPGKGLEWIGHIYYSGSTYYIPSLKSRTTISVDTSKNQFSLKLNSVTAADTAVYYCARGTVTTYYFDYWGQGTTVTVSSASTKGPSVFPPLAPCSRSTST

SEQ ID NO: 55 - protein, 118 aa, Homo sapiens
VSGGSVSSGDYYWSWIRQPPGKGLEWIGHLYYSGNTNYNPSLKSRVTISLDTSKNQFSLKLSSVTAADTAVYYCARDFLTGSFFDYWGQGTLVTVSSASTKGPSVFPPLAPCSRSTST

SEQ ID NO: 56 - protein, 117 aa, Homo sapiens
VSGGSVYSGDYYWSWIRQPPGKGLEWIGYIYYSGSTNYNPSLKSRVTISVDTSKNQFSLKLSSVTAADTAVYYCARDSILGATNYWGQGTLVTVSSASTKGPSVFPPLAPCSRSTST

SEQ ID NO: 57 - protein, 116 aa, Homo sapiens
VSGGSVSSGDYYWTWIRQSPGKGLEWIGHIYYSGNTNYNPSLKSRLTISIDTSKTQFSLKLSSVTAADTAIYYCVRDRVTGAFDIWGQGTMVTSSASTKGPSVFPPLAPCSRSTST

SEQ ID NO: 58 - protein, 467 aa, Mus musculus
MEFGLSWLFLVAILKGVQCEVQLLESGGGLVQPGGSLRLSCAASGFTFSSYAMSWVRQAPGKGLEWVSGITGSGGSTYAADSVKGRFTISRDNSKNTLYLQMNSLRAEDTAVYYCAKDPGTTVIMSWFDPWGQGTLVTVSSASTKGPSVFPLAPCSRSTSESTAALGCLVKDYFPEPVTVSWNSGALTSGVHTFPAVLPSSGLYSLSSVVTVPSSNFGTQTYTCNVDHKPSNTKVDKTVERKCCVECPPCPAPPVAGPSVFLFPPKPKDTLMISRTPEVTCVVVDVSHEDPEVQFNWYVDGVEVHNAKTKPREEQFNSTFRVVSVLTVVHQDWLNGKEYKCKVSNKGLPAPIEKTISKTKGQPREPQVYTLPPSREEMTKNQVSLTCLVKGFYPSDIAVEWESNGQPENNYKTTPPMLDSDGSFFLYSKLTVDKSRWQQGNVFSCSVMHEALHNHYTQKSLSLSPGK

SEQ ID NO: 59 - protein, 235 aa, Mus musculus
METPAQLLFLLLLWLPDTTGEIVLTQSPGTLSLSPGERATLSCRASQSVRGRYLAWYQQKPGQAPRLLIYGASSRATGIPDRFSGSGSGTDFTLTISRLEPEDFAVFRCQQYGSSPRTFGQGTKVEIKRTVAAPSVFIFPPSDEQLKSGTASVVCLLNNFYPREAKVQWKVDNALQSGNSQESVTEQDSKDSTYSLSSTLTLSKADYEKHKVYACEVTHQGLSSPVTKSFNRGEC

SEQ ID NO: 60 - protein, 122 aa, Mus musculus
EVQLLESGGGLVQPGGSLRLSCAASGFTFSSYAMSWVRQAPGKGLEWVSGITGSGGSTYYADSVKGRFTISRDNSKNTLYLQMNSLRAEDTAVYYCAKDPGTTVIMSWFDPWGQGTLVTVSS

SEQ ID NO: 61 - protein, 108 aa, Mus musculus
EIVLTQSPGTLSLSPGERATLSCRASQSVRGRYLAWYQQKPGQAPRLLIYGASSRATGIPDRFSGSGSGTDFTLTISRLEPEDFAVFYCQQYGSSPRTFGQGTKVEIK

SEQ ID NO: 62 - protein, 139 aa, Homo sapiens
MEFGLSWVFLVALLRGVQCQVQLVESGGGVVQPGRSLRLSCAASGFTFSNYGMHWVRQAPGKGLEWVAGIWNDGINKYHAHSVRGRFTISRDNSKNTLYLQMNSPRAEDTAVYYCARARSFDWLLFEFWGQGTLVTVSS

SEQ ID NO: 63 - protein, 128 aa, Homo sapiens
MEAPAQLLFLLLLWLPDTTGEIVLTQSPATLSLSPGERATLSCRASQSVSSYLAWYQQKPGQAPRLLIYDASNRATGIPARFSGSGSGTDFTLTISSLEPEDFAVYYCQQRSNWPPLTFGGGTKVEIK

SEQ ID NO: 64 - protein, 139 aa, Homo sapiens
MEFGLSWVFLVALLRGVQCQVQLVESGGGVVQPGRSLRLSCAVSGFTFSNYGMHWVRQAPGKGLEWVAAIWNDGENKHHAGSVRGRFTISRDNSKNTLYLQMNSLRAEDTAVYYCARGRYFDWLLFEYWGQGTLVTVSS

SEQ ID NO: 65 - protein, 137 aa, Homo sapiens
MGSTAILALLLAVLQGVCAEVQLMQSGAEVKKPGESLKISCKGSGYSFSFHWIAWVRQMPGKGLEWMGIIHPGASDTRYSPSFQGQVTISADNSNSATYLQWSSLKASDTAMYFCARQRELDYFDYWGQGTLVTVSS

SEQ ID NO: 66 - protein, 126 aa, Homo sapiens
MSPSQLIGFLLLWVPASRGEIVLTQSPDFQSVTPKEKVTITCRASQSIGSSLHWYQQKPDQSPKLLIKYASQSFSGVPSRFSGSGSGTDFTLTINSLEAEDAAAYYCHQSSSLPLTFGGGTKVEIK

SEQ ID NO: 67 - protein, 469 aa, Homo sapiens
MEFGLSWVFLVALLRGVQCQVQLVESGGGVVQPGRSLRLSCAASGFTFSNYGMHWVRQAPGKGLEWVAGIWNDGINKYHAHSVRGRFTISRDNSKNTLYLQMNSPRAEDTAVYYCARARSFDWLLFEFWGQGTLVTVSSASTKGPSVFPLAPSSKSTSGGTAALGCLVKDYFPEPVTVSWNSGALTSGVHTFPAVLQSSGLYSLSSVVTVPSSSLGTQTYICNVNHKPSNTKVDKKVEPKSCDKTHTCPPCPAPELLGGPSVFLFPPKPKDTLMISRTPEVTCVVVDVSHEDPEVKFNWYVDGVEVHNAKTKPREEQYNSTYRVVSVLTVLHQDWLNGKEYKCKVSNKALPAPIEKTISKAKGQPREPQVYTLPPSRDELTKNQVSLTCLVKGFYPSDIAVEWESNGQPENNYKTTPPVLDSDGSFFLYSKLTVDKSRWQQGNVFSCSVMHEALHNHYTQKSLSLSPGK

SEQ ID NO: 68 - protein, 465 aa, Homo sapiens
MEFGLSWVFLVALLRGVQCQVQLVESGGGVVQPGRSLRLSCAASGFTFSNYGMHWVRQAPGKGLEWVAGIWNDGINKYHAHSVRGRFTISRDNSKNTLYLQMNSPRAEDTAVYYCARARSFDWLLFEFWGQGTLVTVSSASTKGPSVFPLAPCSRSTSESTAALGCLVKDYFPEPVTVSWNSGALTSGVHTFPAVLQSSGLYSLSSVVTVPSSNFGTQTYTCNVDHKPSNTKVDKTVERKCCVECPPCPAPPVAGPSVFLFPPKPKDTLMISRTPEVTCVVVDVSHEDPEVQFNWYVDGVEVHNAKTKPREEQFNSTFRVVSVLTVVHQDWLNGKEYKCKVSNKGLPAPIEKTISKTKGQPREPQVYTLPPSREEMTKNQVSLTCLVKGFYPSDIAVEWESNGQPENNYKTTPPMLDSDGSFFLYSKLTVDKSRWQQGNVFSCSVMHEALHNHYTQKSLSLSPGK

SEQ ID NO: 69 - protein, 466 aa, Homo sapiens
MEFGLSWVFLVALLRGVQCQVQLVESGGGVVQPGRSLRLSCAASGFTFSNYGMHWVRQAPGKGLEWVAGIWNDGINKYHAHSVRGRFTISRDNSKNTLYLQMNSPRAEDTAVYYCARARSFDWLLFEFWGQGTLVTVSSASTKGPSVFPLAPCSRSTSESTAALGCLVKDYFPEPVTVSWNSGALTSGVHTFPAVLQSSGLYSLSSVVTVPSSSLGTKTYTCNVDHKPSNTKVDKRVESKYGPPCPSCPAPEFEGGPSVFLFPPKPKDTLMISRTPEVTCVVVDVSQEDPEVQFNWYVDGVEVHNAKTKPREEQFNSTYRVVSVLTVLHQDWLNGKEYKCKVSNKGLPSSIEKTISKAKGQPREPQVYTLPPSQEEMTKNQVSLTCLVKGFYPSDIAVEWESNGQPENNYKTTPPVLDSDGSFFLYSRLTVDKSRWQEGNVFSCSVMHEALHNHYTQKSLSLSLGK

SEQ ID NO: 70 - protein, 469 aa, Homo sapiens
MEFGLSWVFLVALLRGVQCQVQLVESGGGVVQPGRSLRLSCAVSGFTFSNYGMHWVRQAPGKGLEWVAAIWNDGENKHHAGSVRGRFTISRDNSKNTLYLQMNSLRAEDTAVYYCARGRYFDWLLFEYWGQGTLVTVSSASTKGPSVFPLAPSSKSTSGGTAALGCLVKDYFPEPVTVSWNSGALTSGVHTFPAVLQSSGLYSLSSVVTVPSSSLGTQTYICNVNHKPSNTKVDKKVEPKSCDKTHTCPPCPAPELLGGPSVFLFPPKPKDTLMISRTPEVTCVVVDVSHEDPEVKFNWYVDGVEVHNAKTKPREEQYNSTYRVVSVLTVLHQDWLNGKEYKCKVSNKALPAPIEKTISKAKGQPREPQVYTLPPSRDELTKNQVSLTCLVKGFYPSDIAVEWESNGQPENNYKTTPPVLDSDGSFFLYSKLTVDKSRWQQGNVFSCSVMHEALHNHYTQKSLSLSPGK

SEQ ID NO: 71 - protein, 465 aa, Homo sapiens
MEFGLSWVFLVALLRGVQCQVQLVESGGGVVQPGRSLRLSCAVSGFTFSNYGMHWVRQAPGKGLEWVAAIWNDGENKHHAGSVRGRFTISRDNSKNTLYLQMNSLRAEDTAVYYCARGRYFDWLLFEYWGQGTLVTVSSASTKGPSVFPLAPCSRSTSESTAALGCLVKDYFPEPVTVSWNSGALTSGVHTFPAVLQSSGLYSLSSVVTVPSSNFGTQTYTCNVDHKPSNTKVDKTVERKCCVECPPCPAPPVAGPSVFLFPPKPKDTLMISRTPEVTCVVVDVSHEDPEVQFNWYVDGVEVHNAKTKPREEQFNSTFRVVSVLTVVHQDWLNGKEYKCKVSNKGLPAPIEKTISKTKGQPREPQVYTLPPSREEMTKNQVSLTCLVKGFYPSDIAVEWESNGQPENNYKTTPPMLDSDGSFFLYSKLTVDKSRWQQGNVFSCSVMHEALHNHYTQKSLSLSPGK

SEQ ID NO: 72 - protein, 466 aa, Homo sapiens
MEFGLSWVFLVALLRGVQCQVQLVESGGGVVQPGRSLRLSCAVSGFTFSNYGMHWVRQAPGKGLEWVAAIWNDGENKHHAGSVRGRFTISRDNSKNTLYLQMNSLRAEDTAVYYCARGRYFDWLLFEYWGQGTLVTVSSASTKGPSVFPLAPCSRSTSESTAALGCLVKDYFPEPVTVSWNSGALTSGVHTFPAVLQSSGLYSLSSVVTVPSSSLGTKTYTCNVDHKPSNTKVDKRVESKYGPPCPSCPAPEFEGGPSVFLFPPKPKDTLMISRTPEVTCVVVDVSQEDPEVQFNWYVDGVEVHNAKTKPREEQFNSTYRVVSVLTVLHQDWLNGKEYKCKVSNKGLPSSIEKTISKAKGQPREPQVYTLPPSQEEMTKNQVSLTCLVKGFYPSDIAVEWESNGQPENNYKTTPPVLDSDGSFFLYSRLTVDKSRWQEGNVFSCSVMHEALHNHYTQKSLSLSLGK

SEQ ID NO: 73 - protein, 467 aa, Homo sapiens
MGSTAILALLLAVLQGVCAEVQLMQSGAEVKKPGESLKISCKGSGYSFSFHWIAWVRQMPGKGLEWMGIIHPGASDTRYSPSFQGQVTISADNSNSATYLQWSSLKASDTAMYFCARQRELDYFDYWGQGTLVTVSSASTKGPSVFPLAPSSKSTSGGTAALGCLVKDYFPEPVTVSWNSGALTSGVHTFPAVLQSSGLYSLSSVVTVPSSSLGTQTYICNVNHKPSNTKVDKKVEPKSCDKTHTCPPCPAPELLGGPSVFLFPPKPKDTLMISRTPEVTCVVVDVSHEDPEVKFNWYVDGVEVHNAKTKPREEQYNSTYRVVSVLTVLHQDWLNGKEYKCKVSNKALPAPIEKTISKAKGQPREPQVYTLPPSRDELTKNQVSLTCLVKGFYPSDIAVEWESNGQPENNYKTTPPVLDSDGSFFLYSKLTVDKSRWQQGNVFSCSVMHEALHNHYTQKSLSLSPGK

SEQ ID NO: 74 - protein, 463 aa, Homo sapiens
MGSTAILALLLAVLQGVCAEVQLMQSGAEVKKPGESLKISCKGSGYSFSFHWIAWVRQMPGKGLEWMGIIHPGASDTRYSPSFQGQVTISADNSNSATYLQWSSLKASDTAMYFCARQRELDYFDYWGQGTLVTVSSASTKGPSVFPLAPCSRSTSESTAALGCLVKDYFPEPVTVSWNSGALTSGVHTFPAVLQSSGLYSLSSVVTVPSSNFGTQTYTCNVDHKPSNTKVDKTVERKCCVECPPCPAPPVAGPSVFLFPPKPKDTLMISRTPEVTCVVVDVSHEDPEVQFNWYVDGVEVHNAKTKPREEQFNSTFRVVSVLTVVHQDWLNGKEYKCKVSNKGLPAPIEKTISKTKGQPREPQVYTLPPSREEMTKNQVSLTCLVKGFYPSDIAVEWESNGQPENNYKTTPPMLDSDGSFFLYSKLTVDKSRWQQGNVFSCSVMHEALHNHYTQKSLSLSPGK

SEQ ID NO: 75 - protein, 464 aa, Homo sapiens
MGSTAILALLLAVLQGVCAEVQLMQSGAEVKKPGESLKISCKGSGYSFSFHWIAWVRQMPGKGLEWMGIIHPGASDTRYSPSFQGQVTISADNSNSATYLQWSSLKASDTAMYFCARQRELDYFDYWGQGTLVTVSSASTKGPSVFPLAPCSRSTSESTAALGCLVKDYFPEPVTVSWNSGALTSGVHTFPAVLQSSGLYSLSSVVTVPSSSLGTKTYTCNVDHKPSNTKVDKRVESKYGPPCPSCPAPEFEGGPSVFLFPPKPKDTLMISRTPEVTCVVVDVSQEDPEVQFNWYVDGVEVHNAKTKPREEQFNSTYRVVSVLTVLHQDWLNGKEYKCKVSNKGLPSSIEKTISKAKGQPREPQVYTLPPSQEEMTKNQVSLTCLVKGFYPSDIAVEWESNGQPENNYKTTPPVLDSDGSFFLYSRLTVDKSRWQEGNVFSCSVMHEALHNHYTQKSLSLSLGK

SEQ ID NO: 76 - protein, 235 aa, Homo sapiens
MEAPAQLLFLLLLWLPDTTGEIVLTQSPATLSLSPGERATLSCRASQSVSSYLAWYQQKPGQAPRLLIYDASNRATGIPARFSGSGSGTDFTLTISSLEPEDFAVYYCQQRSNWPPLTFGGGTKVEIKRTVAAPSVFIFPPSDEQLKSGTASVVCLLNNFYPREAKVQWKVDNALQSGNSQESVTEQDSKDSTYSLSSTLTLSKADYEKHKVYACEVTHQGLSSPVTKSFNRGEC

SEQ ID NO: 77 - protein, 233 aa, Homo sapiens
MSPSQLIGFLLLWVPASRGEIVLTQSPDFQSVTPKEKVTITCRASQSIGSSLHWYQQKPDQSPKLLIKYASQSFSGVPSRFSGSGSGTDFTLTINSLEAEDAAAYYCHQSSSLPLTFGGGTKVEIKRTVAAPSVFIFPPSDEQLKSGTASVVCLLNNFYPREAKVQWKVDNALQSGNSQESVTEQDSKDSTYSLSSTLTLSKADYEKHKVYACEVTHQGLSSPVTKSFNRGEC

SEQ ID NO: 78 - protein, 120 aa, Homo sapiens
QVQLVESGGGVVQPGRSLRLSCAASGFTFSNYGMHWVRQAPGKGLEWVAGIWNDGINKYHAHSVRGRFTISRDNSKNTLYLQMNSPRAEDTAVYYCARARSFDWLLFEFWGQGTLVTVSS

SEQ ID NO: 79 - protein, 109 aa, Homo sapiens
GEIVLTQSPATLSLSPGERATLSCRASQSVSSYLAWYQQKPGQAPRLLIYDASNRATGIPARFSGSGSGTDFTLTISSLEPEDFAVYYCQQRSNWPPLTFGGGTKVEIK

SEQ ID NO: 80 - protein, 120 aa, Homo sapiens
QVQLVESGGGVVQPGRSLRLSCAVSGFTFSNYGMHWVRQAPGKGLEWVAAIWNDGENKHHAGSVRGRFTISRDNSKNTLYLQMNSLRAEDTAVYYCARGRYFDWLLFEYWGQGTLVTVSS

SEQ ID NO: 81 - protein, 118 aa, Homo sapiens
EVQLMQSGAEVKKPGESLKISCKGSGYSFSFHWIAWVRQMPGKGLEWMGIIHPGASDTRYSPSFQGQVTISADNSNSATYLQWSSLKASDTAMYFCARQRELDYFDYWGQGTLVTVSS

SEQ ID NO: 82 - protein, 107 aa, Homo sapiens
EIVLTQSPDFQSVTPKEKVTITCRASQSIGSSLHWYQQKPDQSPKLLIKYASQSFSGVPSRFSGSGSGTDFTLTINSLEAEDAAAYYCHQSSSLPLTFGGGTKVEIK

SEQ ID NO: 83 - protein, 11 aa, Homo sapiens
RKCACVECPPC

SEQ ID NO: 84 - protein, 12 aa, Homo sapiens
RKCPPCVECPPC

SEQ ID NO: 85 - protein, 12 aa, Homo sapiens
RKANCCVECPPC

SEQ ID NO: 86 - protein, 12 aa, Homo sapiens
RKPNCCVECPPC